European Patent Application EP 4 151 232 A1, published March 22, 2023. Title: VACUNA RECOMBINANTE CONTRA COVID-19 EN VECTOR VIRAL DE PARAMIXOVIRUS. Applicant: Laboratorio Avi-Mex S.A. de C.V. The sequence listing filed with the application follows.

SEQUENCE LISTING (14 sequences)

SEQ ID NO: 1 - DNA, 3870 bp, SARS-CoV2
ccgcggttagaaaaaatacgggtagaaccgccaccatgtttgtttttcttgttttattgccactagtctctagtcagtgtgttaatcttacaaccagaactcaattaccccctgcatacactaattctttcacacgtggtgtttattaccctgacaaagttttcagatcctcagttttacattcaactcaggacttgttcttacctttcttttccaatgttacttggttccatgctatacatgtctctgggaccaatggtactaagaggtttgataaccctgtcctaccatttaatgatggtgtttattttgcttccactgagaagtctaacataataagaggctggatttttggtactactttagattcgaagacccagtccctacttattgttaataacgctactaatgttgttattaaagtctgtgaatttcaattttgtaatgatccatttttgggtgtttattaccacaagaacaacaaaagttggatggaaagtgagttcagagtttattctagtgcgaataattgcacttttgaatatgtctctcagccttttcttatggaccttgaaggaaaacagggtaatttcaagaatcttagggaatttgtgtttaagaatattgatggttattttaaaatatattctaagcacacgcctattaatttagtgcgtgatctccctcagggtttttcggctttagaaccattggtagatttgccaataggtattaacatcactaggtttcaaactttacttgctttacatagaagttatttgactcctggtgattcttcttcaggttggacagctggtgctgcagcttattatgtgggttatcttcaacctaggacttttctattaaaatataatgaaaatggaaccattacagatgctgtagactgtgcacttgaccctctctcagaaacaaagtgtacgttgaaatccttcactgtagagaaaggaatctatcaaacttctaactttagagtccaaccaacagaatctattgttagatttcctaatattacaaacttgtgcccttttggtgaagtttttaacgccaccagatttgcatctgtttatgcttggaacaggaagagaatcagcaactgtgttgctgattattctgtcctatataattccgcatcattttccacttttaagtgttatggagtgtctcctactaaattaaatgatctctgctttactaatgtctatgcagattcatttgtaattagaggtgatgaagtcagacaaatcgctccagggcaaactggaaagattgctgattataattataaattaccagatgattttacaggctgcgttatagcttggaattctaacaatcttgattctaaggttggtggtaattataattacctgtatagattgtttaggaagtctaatctcaaaccttttgagagagatatttcaactgaaatctatcaggccggtagcacaccttgtaatggtgttgaaggttttaattgttactttcctttacaatcatatggtttccaacccactaatggtgttggttaccaaccatacagagtagtagtactttcttttgaacttctacatgcaccagcaactgtttgtggacctaagaagtctactaatttggttaagaacaaatgtgtcaatttcaacttcaatggtttaacaggcacaggtgttcttactgagtctaacaagaagtttctgcctttccaacaatttggcagagacattgctgacactactgatgctgtccgtgatccacagacacttgagattcttgacattacaccatgttcttttggtggtgtcagtgttataacaccaggaacaaatacttctaaccaggttgctgttctttatcaggatgttaactgcacagaagtccctgttgctattcatgcagatcaacttactcctacttggcgtgtttattctacaggttctaatgtttttcaaacacgtgcaggctgtttaataggggctgaacatgtcaacaactcatatgagtgtgacatacccattggtgcaggtatatgcgctagttatcagactcagactaattctcctcggcgggcacgtagtgtagctagtcaatccatcattgcctacactatgtcacttggtgcagaaaattcagttgcttactctaataactctattgccatacccacaaattttactattagtgttaccacagaaattctaccagtgtctatgaccaagacatcagtagattgtacaatgtacatttgtggtgattcaactgaatgcagcaatcttttgttgcaatatggcagtttttgtacacaattaaaccgtgctttaactggaatagctgttgaacaagacaagaacacccaagaagtttttgcacaagtcaaacaaatttacaaaacaccaccaattaaagattttggtggttttaatttttcacaaatattaccagatccatcaaaaccaagcaagaggtcatttattgaagatctacttttcaacaaagtgacacttgcagatgctggcttcatcaaacaatatggtgattgccttggtgatattgctgctagagacctcatttgtgcacaaaagtttaacggccttactgttttgccacctttgctcacagatgaaatgattgctcaatacacttctgcactgttagcgggtacaatcacttctggttggacctttggtgcaggtgctgcattacaaataccatttgctatgcaaatggcttataggtttaatggtattggagttacacagaatgttctctatgagaaccagaaattgattgccaaccaatttaatagtgctattggcaaaattcaagactcactttcttccacagcaagtgcacttggaaaacttcaagatgtggtcaaccaaaatgcacaagctttaaacacgcttgttaaacaacttagctccaattttggtgcaatttcaagtgttttaaatgatatcctttcacgtcttgacaaagttgaggctgaagtgcaaattgataggttgatcacaggcagacttcaaagtttgcagacatatgtgactcaacaattaattagagctgcagaaatcagagcttctgctaatcttgctgctactaaaatgtcagagtgtgtacttggacaatcaaagagagttgatttttgtggaaagggctatcatcttatgtccttccctcagtcagcacctcatggtgtagtcttcttgcatgtgacttatgtccctgcacaagaaaagaacttcacaactgctcctgccatttgtcatgatggaaaagcacactttcctcgtgaaggtgtctttgtttcaaatggcacacactggtttgtaacacaaaggaatttttatgaaccacaaatcattactacagacaacacatttgtgtctggtaactgtgatgttgtaataggaattgtcaacaacacagtttatgatcctttgcaacctgaattagactcattcaaggaggagttagataaatattttaagaatcatacatcaccagatgttgatttaggtgacatctctggcattaatgcttcagttgtaaacattcagaaagaaattgaccgcctcaatgaggttgccaagaatttaaatgaatctctcatcgatctccaagaacttggaaagtatgagcagtatataaaatggccatggtacatttggctaggttttatagctggcttgattgccatagtaatggtgacaattatgctttgctgtatgaccagttgctgtagttgtctcaagggctgttgttcttgtggatcctgctgcaaatttgatgaagacgactctgagccagtgctcaaaggagtcaaattacattacacataataatgaaccgcgg

SEQ ID NO: 2 - DNA, 2268 bp, SARS-CoV2
ccgcggttagaaaaaatacgggtagaaccgccaccatgtttgtttttcttgttttattgccactagtctctagtcagtgtgttaatcttacaaccagaactcaattaccccctgcatacactaattctttcacacgtggtgtttattaccctgacaaagttttcagatcctcagttttacattcaactcaggacttgttcttacctttcttttccaatgttacttggttccatgctatacatgtctctgggaccaatggtactaagaggtttgataaccctgtcctaccatttaatgatggtgtttattttgcttccactgagaagtctaacataataagaggctggatttttggtactactttagattcgaagacccagtccctacttattgttaataacgctactaatgttgttattaaagtctgtgaatttcaattttgtaatgatccatttttgggtgtttattaccacaagaacaacaaaagttggatggaaagtgagttcagagtttattctagtgcgaataattgcacttttgaatatgtctctcagccttttcttatggaccttgaaggaaaacagggtaatttcaagaatcttagggaatttgtgtttaagaatattgatggttattttaaaatatattctaagcacacgcctattaatttagtgcgtgatctccctcagggtttttcggctttagaaccattggtagatttgccaataggtattaacatcactaggtttcaaactttacttgctttacatagaagttatttgactcctggtgattcttcttcaggttggacagctggtgctgcagcttattatgtgggttatcttcaacctaggacttttctattaaaatataatgaaaatggaaccattacagatgctgtagactgtgcacttgaccctctctcagaaacaaagtgtacgttgaaatccttcactgtagagaaaggaatctatcaaacttctaactttagagtccaaccaacagaatctattgttagatttcctaatattacaaacttgtgcccttttggtgaagtttttaacgccaccagatttgcatctgtttatgcttggaacaggaagagaatcagcaactgtgttgctgattattctgtcctatataattccgcatcattttccacttttaagtgttatggagtgtctcctactaaattaaatgatctctgctttactaatgtctatgcagattcatttgtaattagaggtgatgaagtcagacaaatcgctccagggcaaactggaaagattgctgattataattataaattaccagatgattttacaggctgcgttatagcttggaattctaacaatcttgattctaaggttggtggtaattataattacctgtatagattgtttaggaagtctaatctcaaaccttttgagagagatatttcaactgaaatctatcaggccggtagcacaccttgtaatggtgttgaaggttttaattgttactttcctttacaatcatatggtttccaacccactaatggtgttggttaccaaccatacagagtagtagtactttcttttgaacttctacatgcaccagcaactgtttgtggacctaagaagtctactaatttggttaagaacaaatgtgtcaatttcaacttcaatggtttaacaggcacaggtgttcttactgagtctaacaagaagtttctgcctttccaacaatttggcagagacattgctgacactactgatgctgtccgtgatccacagacacttgagattcttgacattacaccatgttcttttggtggtgtcagtgttataacaccaggaacaaatacttctaaccaggttgctgttctttatcaggatgttaactgcacagaagtccctgttgctattcatgcagatcaacttactcctacttggcgtgtttattctacaggttctaatgtttttcaaacacgtgcaggctgtttaataggggctgaacatgtcaacaactcatatgagtgtgacatacccattggtgcaggtatatgcgctagttatcagactcagactaattctcctcggcgggcacgtgttaacctcattacctatatcgttttgactatcatatctcttgtttttggtatacttagcctgattctagcatgctacctaatgtacaagcaaaaggcgcaacaaaagaccttattatggcttgggaataataccctagatcagatgagagccactacaaagatgtaatgaaccgcgg

SEQ ID NO: 3 - DNA, 3852 bp, SARS-CoV2
ccgcggttagaaaaaatacgggtagaaccgccaccatgtttgtttttcttgttttattgccactagtctctagtcagtgtgttaatcttacaaccagaactcaattaccccctgcatacactaattctttcacacgtggtgtttattaccctgacaaagttttcagatcctcagttttacattcaactcaggacttgttcttacctttcttttccaatgttacttggttccatgctatacatgtctctgggaccaatggtactaagaggtttgataaccctgtcctaccatttaatgatggtgtttattttgcttccactgagaagtctaacataataagaggctggatttttggtactactttagattcgaagacccagtccctacttattgttaataacgctactaatgttgttattaaagtctgtgaatttcaattttgtaatgatccatttttgggtgtttattaccacaagaacaacaaaagttggatggaaagtgagttcagagtttattctagtgcgaataattgcacttttgaatatgtctctcagccttttcttatggaccttgaaggaaaacagggtaatttcaagaatcttagggaatttgtgtttaagaatattgatggttattttaaaatatattctaagcacacgcctattaatttagtgcgtgatctccctcagggtttttcggctttagaaccattggtagatttgccaataggtattaacatcactaggtttcaaactttacttgctttacatagaagttatttgactcctggtgattcttcttcaggttggacagctggtgctgcagcttattatgtgggttatcttcaacctaggacttttctattaaaatataatgaaaatggaaccattacagatgctgtagactgtgcacttgaccctctctcagaaacaaagtgtacgttgaaatccttcactgtagagaaaggaatctatcaaacttctaactttagagtccaaccaacagaatctattgttagatttcctaatattacaaacttgtgcccttttggtgaagtttttaacgccaccagatttgcatctgtttatgcttggaacaggaagagaatcagcaactgtgttgctgattattctgtcctatataattccgcatcattttccacttttaagtgttatggagtgtctcctactaaattaaatgatctctgctttactaatgtctatgcagattcatttgtaattagaggtgatgaagtcagacaaatcgctccagggcaaactggaaagattgctgattataattataaattaccagatgattttacaggctgcgttatagcttggaattctaacaatcttgattctaaggttggtggtaattataattacctgtatagattgtttaggaagtctaatctcaaaccttttgagagagatatttcaactgaaatctatcaggccggtagcacaccttgtaatggtgttgaaggttttaattgttactttcctttacaatcatatggtttccaacccactaatggtgttggttaccaaccatacagagtagtagtactttcttttgaacttctacatgcaccagcaactgtttgtggacctaagaagtctactaatttggttaagaacaaatgtgtcaatttcaacttcaatggtttaacaggcacaggtgttcttactgagtctaacaagaagtttctgcctttccaacaatttggcagagacattgctgacactactgatgctgtccgtgatccacagacacttgagattcttgacattacaccatgttcttttggtggtgtcagtgttataacaccaggaacaaatacttctaaccaggttgctgttctttatcaggatgttaactgcacagaagtccctgttgctattcatgcagatcaacttactcctacttggcgtgtttattctacaggttctaatgtttttcaaacacgtgcaggctgtttaataggggctgaacatgtcaacaactcatatgagtgtgacatacccattggtgcaggtatatgcgctagttatcagactcagactaattctcctcggcgggcacgtagtgtagctagtcaatccatcattgcctacactatgtcacttggtgcagaaaattcagttgcttactctaataactctattgccatacccacaaattttactattagtgttaccacagaaattctaccagtgtctatgaccaagacatcagtagattgtacaatgtacatttgtggtgattcaactgaatgcagcaatcttttgttgcaatatggcagtttttgtacacaattaaaccgtgctttaactggaatagctgttgaacaagacaagaacacccaagaagtttttgcacaagtcaaacaaatttacaaaacaccaccaattaaagattttggtggttttaatttttcacaaatattaccagatccatcaaaaccaagcaagaggtcatttattgaagatctacttttcaacaaagtgacacttgcagatgctggcttcatcaaacaatatggtgattgccttggtgatattgctgctagagacctcatttgtgcacaaaagtttaacggccttactgttttgccacctttgctcacagatgaaatgattgctcaatacacttctgcactgttagcgggtacaatcacttctggttggacctttggtgcaggtgctgcattacaaataccatttgctatgcaaatggcttataggtttaatggtattggagttacacagaatgttctctatgagaaccagaaattgattgccaaccaatttaatagtgctattggcaaaattcaagactcactttcttccacagcaagtgcacttggaaaacttcaagatgtggtcaaccaaaatgcacaagctttaaacacgcttgttaaacaacttagctccaattttggtgcaatttcaagtgttttaaatgatatcctttcacgtcttgacaaagttgaggctgaagtgcaaattgataggttgatcacaggcagacttcaaagtttgcagacatatgtgactcaacaattaattagagctgcagaaatcagagcttctgctaatcttgctgctactaaaatgtcagagtgtgtacttggacaatcaaagagagttgatttttgtggaaagggctatcatcttatgtccttccctcagtcagcacctcatggtgtagtcttcttgcatgtgacttatgtccctgcacaagaaaagaacttcacaactgctcctgccatttgtcatgatggaaaagcacactttcctcgtgaaggtgtctttgtttcaaatggcacacactggtttgtaacacaaaggaatttttatgaaccacaaatcattactacagacaacacatttgtgtctggtaactgtgatgttgtaataggaattgtcaacaacacagtttatgatcctttgcaacctgaattagactcattcaaggaggagttagataaatattttaagaatcatacatcaccagatgttgatttaggtgacatctctggcattaatgcttcagttgtaaacattcagaaagaaattgaccgcctcaatgaggttgccaagaatttaaatgaatctctcatcgatctccaagaacttggaaagtatgagcagtatataaaatggccagttaacctcattacctatatcgttttgactatcatatctcttgtttttggtatacttagcctgattctagcatgctacctaatgtacaagcaaaaggcgcaacaaaagaccttattatggcttgggaataataccctagatcagatgagagccactacaaagatgtaatgaaccgcgg

SEQ ID NO: 4 - DNA, 3858 bp, SARS-CoV2
ccgcggttagaaaaaatacgggtagaaccgccaccatgttcgtgtttctggtgctgctgcctctggtgtccagccagtgtgtgaacctgaccacaagaacccagctgcctccagcctacaccaacagctttaccagaggcgtgtactaccccgacaaggtgttcagatccagcgtgctgcactctacccaggacctgttcctgcctttcttcagcaacgtgacctggttccacgccatccacgtgtccggcaccaatggcaccaagagattcgacaaccccgtgctgcccttcaacgacggggtgtactttgccagcaccgagaagtccaacatcatcagaggctggatcttcggcaccacactggacagcaagacccagagcctgctgatcgtgaacaacgccaccaacgtggtcatcaaagtgtgcgagttccagttctgcaacgaccccttcctgggcgtctactatcacaagaacaacaagagctggatggaaagcgagttccgggtgtacagcagcgccaacaactgcaccttcgagtacgtgtcccagcctttcctgatggacctggaaggcaagcagggcaacttcaagaacctgcgcgagttcgtgttcaagaacatcgacggctacttcaagatctacagcaagcacacccctatcaacctcgtgcgggatctgcctcagggcttctctgctctggaacccctggtggatctgcccatcggcatcaacatcacccggtttcagacactgctggccctgcacagaagctacctgacacctggcgatagcagcagcggatggacagctggtgccgccgcttactatgtgggctacctgcagcctagaacctttctgctgaagtacaacgagaacggcaccatcaccgacgccgtggattgtgctctggatcctctgagcgagacaaagtgcaccctgaagtccttcaccgtggaaaagggcatctaccagaccagcaacttccgggtgcagcccaccgaatccatcgtgcggttccccaatatcaccaatctgtgccccttcggcgaggtgttcaatgccaccagattcgcctctgtgtacgcctggaaccggaagcggatcagcaattgcgtggccgactactccgtgctgtacaactccgccagcttcagcaccttcaagtgctacggcgtgtcccctaccaagctgaacgacctgtgcttcacaaacgtgtacgccgacagcttcgtgatccggggagatgaagtgcggcagattgcccctggacagacaggcaagatcgccgactacaactacaagctgcccgacgacttcaccggctgtgtgattgcctggaacagcaacaacctggactccaaagtcggcggcaactacaattacctgtaccggctgttccggaagtccaatctgaagcccttcgagcgggacatctccaccgagatctatcaggccggcagcaccccttgtaacggcgtggaaggcttcaactgctacttcccactgcagtcctacggctttcagcccacaaatggcgtgggctatcagccctacagagtggtggtgctgagcttcgaactgctgcatgcccctgccacagtgtgcggccctaagaaaagcaccaatctcgtgaagaacaaatgcgtgaacttcaacttcaacggcctgaccggcaccggcgtgctgacagagagcaacaagaagttcctgccattccagcagtttggccgggatatcgccgataccacagacgccgttagagatccccagacactggaaatcctggacatcaccccttgcagcttcggcggagtgtctgtgatcacccctggcaccaacaccagcaatcaggtggcagtgctgtaccaggacgtgaactgtaccgaagtgcccgtggccattcacgccgatcagctgacacctacatggcgggtgtactccaccggcagcaatgtgtttcagaccagagccggctgtctgatcggagccgagcacgtgaacaatagctacgagtgcgacatccccatcggcgctggcatctgtgccagctaccagacacagacaaacagccccgcctctgtggccagccagagcatcattgcctacacaatgtctctgggcgccgagaacagcgtggcctactccaacaactctatcgctatccccaccaacttcaccatcagcgtgaccacagagatcctgcctgtgtccatgaccaagaccagcgtggactgcaccatgtacatctgcggcgattccaccgagtgctccaacctgctgctgcagtacggcagcttctgcacccagctgaatagagccctgacagggatcgccgtggaacaggacaagaacacccaagaggtgttcgcccaagtgaagcagatctacaagacccctcctatcaaggacttcggcggcttcaatttcagccagattctgcccgatcctagcaagcccagcaagcggagcttcatcgaggacctgctgttcaacaaagtgacactggccgacgccggcttcatcaagcagtatggcgattgtctgggcgacattgccgccagggatctgatttgcgcccagaagtttaacggactgacagtgctgcctcctctgctgaccgatgagatgatcgcccagtacacatctgccctgctggccggcacaatcacaagcggctggacatttggagctggcgccgctctgcagatcccctttgctatgcagatggcctaccggttcaacggcatcggagtgacccagaatgtgctgtacgagaaccagaagctgatcgccaaccagttcaacagcgccatcggcaagatccaggacagcctgagcagcacagcaagcgccctgggaaagctgcaggacgtggtcaaccagaatgcccaggcactgaacaccctggtcaagcagctgtcctccaacttcggcgccatcagctctgtgctgaacgatatcctgagcagactggaccctcctgaagccgaggtgcagatcgacagactgatcaccggaaggctgcagtccctgcagacctacgttacccagcagctgatcagagccgccgagattagagcctctgccaatctggccgccaccaagatgtctgagtgtgtgctgggccagagcaagagagtggacttttgcggcaagggctaccacctgatgagcttccctcagtctgcccctcacggcgtggtgtttctgcacgtgacatacgtgcccgctcaagagaagaatttcaccaccgctccagccatctgccacgacggcaaagcccactttcctagagaaggcgtgttcgtgtccaacggcacccattggttcgtgacccagcggaacttctacgagccccagatcatcaccaccgacaacaccttcgtgtctggcaactgcgacgtcgtgatcggcattgtgaacaataccgtgtacgaccctctgcagcccgagctggacagcttcaaagaggaactggataagtactttaagaaccacacaagccccgacgtggacctgggcgatatcagcggaatcaatgccagcgtcgtgaacatccagaaagagatcgaccggctgaacgaggtggccaagaatctgaacgagagcctgatcgacctgcaagaactggggaagtacgagcagtacatcaagtggccctggtacatttggctaggttttatagctggcttgattgccatagtaatggtgacaattatgctttgctgtatgaccagttgctgtagttgtctcaagggctgttgttcttgtggatcctgctgcaaatttgatgaagacgactctgagccagtgctcaaaggagtcaaattacattacacataatgaaccgcgg

SEQ ID NO: 5 - DNA, 3840 bp, SARS-CoV2
ccgcggttagaaaaaatacgggtagaaccgccaccatgttcgtgtttctggtgctgctgcctctggtgtccagccagtgtgtgaacctgaccacaagaacccagctgcctccagcctacaccaacagctttaccagaggcgtgtactaccccgacaaggtgttcagatccagcgtgctgcactctacccaggacctgttcctgcctttcttcagcaacgtgacctggttccacgccatccacgtgtccggcaccaatggcaccaagagattcgacaaccccgtgctgcccttcaacgacggggtgtactttgccagcaccgagaagtccaacatcatcagaggctggatcttcggcaccacactggacagcaagacccagagcctgctgatcgtgaacaacgccaccaacgtggtcatcaaagtgtgcgagttccagttctgcaacgaccccttcctgggcgtctactatcacaagaacaacaagagctggatggaaagcgagttccgggtgtacagcagcgccaacaactgcaccttcgagtacgtgtcccagcctttcctgatggacctggaaggcaagcagggcaacttcaagaacctgcgcgagttcgtgttcaagaacatcgacggctacttcaagatctacagcaagcacacccctatcaacctcgtgcgggatctgcctcagggcttctctgctctggaacccctggtggatctgcccatcggcatcaacatcacccggtttcagacactgctggccctgcacagaagctacctgacacctggcgatagcagcagcggatggacagctggtgccgccgcttactatgtgggctacctgcagcctagaacctttctgctgaagtacaacgagaacggcaccatcaccgacgccgtggattgtgctctggatcctctgagcgagacaaagtgcaccctgaagtccttcaccgtggaaaagggcatctaccagaccagcaacttccgggtgcagcccaccgaatccatcgtgcggttccccaatatcaccaatctgtgccccttcggcgaggtgttcaatgccaccagattcgcctctgtgtagatcagcaattgcgtggccgactactccgtgctgtacaactccgccagcttcagcaccttcaagtgctacggcgtgtcccctaccaagctgaacgacctgtgcttcacaaacgtgtacgccgacagcttcgtgatccggggagatgaagtgcggcagattgcccctggacagacaggcaagatcgccgactacaactacaagctgcccgacgacttcaccggctgtgtgattgcctggaacagcaacaacctggactccaaagtcggcggcaactacaattacctgtaccggctgttccggaagtccaatctgaagcccttcgagcgggacatctccaccgagatctatcaggccggcagcaccccttgtaacggcgtggaaggcttcaactgctacttcccactgcagtcctacggctttcagcccacaaatggcgtgggctatcagccctacagagtggtggtgctgagcttcgaactgctgcatgcccctgccacagtgtgcggccctaagaaaagcaccaatctcgtgaagaacaaatgcgtgaacttcaacttcaacggcctgaccggcaccggcgtgctgacagagagcaacaagaagttcctgccattccagcagtttggccgggatatcgccgataccacagacgccgttagagatccccagacactggaaatcctggacatcaccccttgcagcttcggcggagtgtctgtgatcacccctggcaccaacaccagcaatcaggtggcagtgctgtaccaggacgtgaactgtaccgaagtgcccgtggccattcacgccgatcagctgacacctacatggcgggtgtactccaccggcagcaatgtgtttcagaccagagccggctgtctgatcggagccgagcacgtgaacaatagctacgagtgcgacatccccatcggcgctggcatctgtgccagctaccagacacagacaaacagccccgcctctgtggccagccagagcatcattgcctacacaatgtctctgggcgccgagaacagcgtggcctactccaacaactctatcgctatccccaccaacttcaccatcagcgtgaccacagagatcctgcctgtgtccatgaccaagaccagcgtggactgcaccatgtacatctgcggcgattccaccgagtgctccaacctgctgctgcagtacggcagcttctgcacccagctgaatagagccctgacagggatcgccgtggaacaggacaagaacacccaagaggtgttcgcccaagtgaagcagatctacaagacccctcctatcaaggacttcggcggcttcaatttcagccagattctgcccgatcctagcaagcccagcaagcggagcttcatcgaggacctgctgttcaacaaagtgacactggccgacgccggcttcatcaagcagtatggcgattgtctgggcgacattgccgccagggatctgatttgcgcccagaagtttaacggactgacagtgctgcctcctctgctgaccgatgagatgatcgcccagtacacatctgccctgctggccggcacaatcacaagcggctggacatttggagctggcgccgctctgcagatcccctttgctatgcagatggcctaccggttcaacggcatcggagtgacccagaatgtgctgtacgagaaccagaagctgatcgccaaccagttcaacagcgccatcggcaagatccaggacagcctgagcagcacagcaagcgccctgggaaagctgcaggacgtggtcaaccagaatgcccaggcactgaacaccctggtcaagcagctgtcctccaacttcggcgccatcagctctgtgctgaacgatatcctgagcagactggaccctcctgaagccgaggtgcagatcgacagactgatcaccggaaggctgcagtccctgcagacctacgttacccagcagctgatcagagccgccgagattagagcctctgccaatctggccgccaccaagatgtctgagtgtgtgctgggccagagcaagagagtggacttttgcggcaagggctaccacctgatgagcttccctcagtctgcccctcacggcgtggtgtttctgcacgtgacatacgtgcccgctcaagagaagaatttcaccaccgctccagccatctgccacgacggcaaagcccactttcctagagaaggcgtgttcgtgtccaacggcacccattggttcgtgacccagcggaacttctacgagccccagatcatcaccaccgacaacaccttcgtgtctggcaactgcgacgtcgtgatcggcattgtgaacaataccgtgtacgaccctctgcagcccgagctggacagcttcaaagaggaactggataagtactttaagaaccacacaagccccgacgtggacctgggcgatatcagcggaatcaatgccagcgtcgtgaacatccagaaagagatcgaccggctgaacgaggtggccaagaatctgaacgagagcctgatcgacctgcaagaactggggaagtacgagcagtacatcaagtggccctggtacatttggctaggttttatagctggcttgattgccatagtaatggtgacaattatgctttgctgtatgaccagttgctgtagttgtctcaagggctgttgttcttgtggatcctgctgcaaatttgatgaagacgactctgagccagtgctcaaaggagtcaaattacattacacataatgaaccgcgg

SEQ ID NO: 6 - DNA, 18394 bp, NDV LaSota
tcttccgcttcctcgctcactgactcgctgcgctcggtcgttcggctgcggcgagcggtatcagctcactcaaaggcggtaatacggttatccacagaatcaggggataacgcaggaaagaacatgtgagcaaaaggccagcaaaaggccaggaaccgtaaaaaggccgcgttgctggcgtttttccataggctccgcccccctgacgagcatcacaaaaatcgacgctcaagtcagaggtggcgaaacccgacaggactataaagataccaggcgtttccccctggaagctccctcgtgcgctctcctgttccgaccctgccgcttaccggatacctgtccgcctttctcccttcgggaagcgtggcgctttctcatagctcacgctgtaggtatctcagttcggtgtaggtcgttcgctccaagctgggctgtgtgcacgaaccccccgttcagcccgaccgctgcgccttatccggtaactatcgtcttgagtccaacccggtaagacacgacttatcgccactggcagcagccactggtaacaggattagcagagcgaggtatgtaggcggtgctacagagttcttgaagtggtggcctaactacggctacactagaagaacagtatttggtatctgcgctctgctgaagccagttaccttcggaaaaagagttggtagctcttgatccggcaaacaaaccaccgctggtagcggtggtttttttgtttgcaagcagcagattacgcgcagaaaaaaaggatctcaagaagatcctttgatcttttctacggggtctgacgctcagtggaacgaaaactcacgttaagggattttggtcatgagattatcaaaaaggatcttcacctagatccttttaaattaaaaatgaagttttaaatcaatctaaagtatatatgagtaaacttggtctgacagttaccaatgcttaatcagtgaggcacctatctcagcgatctgtctatttcgttcatccatagttgcctgactccccgtcgtgtagataactacgatacgggagggcttaccatctggccccagtgctgcaatgataccgcgagacccacgctcaccggctccagatttatcagcaataaaccagccagccggaagggccgagcgcagaagtggtcctgcaactttatccgcctccatccagtctattaattgttgccgggaagctagagtaagtagttcgccagttaatagtttgcgcaacgttgttgccattgctacaggcatcgtggtgtcacgctcgtcgtttggtatggcttcattcagctccggttcccaacgatcaaggcgagttacatgatcccccatgttgtgcaaaaaagcggttagctccttcggtcctccgatcgttgtcagaagtaagttggccgcagtgttatcactcatggttatggcagcactgcataattctcttactgtcatgccatccgtaagatgcttttctgtgactggtgagtactcaaccaagtcattctgagaatagtgtatgcggcgaccgagttgctcttgcccggcgtcaatacgggataataccgcgccacatagcagaactttaaaagtgctcatcattggaaaacgttcttcggggcgaaaactctcaaggatcttaccgctgttgagatccagttcgatgtaacccactcgtgcacccaactgatcttcagcatcttttactttcaccagcgtttctgggtgagcaaaaacaggaaggcaaaatgccgcaaaaaagggaataagggcgacacggaaatgttgaatactcatactcttcctttttcaatattattgaagcatttatcagggttattgtctcatgagcggatacatatttgaatgtatttagaaaaataaacaaataggggttccgcgcacatttccccgaaaagtgccacctgacgtctaagaaaccattattatcatgacattaacctataaaaataggcgtatcacgaggccctttcgtctcgcgcgtttcggtgatgacggtgaaaacctctgacacatgcagctcccggagacggtcacagcttgtctgtaagcggatgccgggagcagacaagcccgtcagggcgcgtcagcgggtgttggcgggtgtcggggctggcttaactatgcggcatcagagcagattgtactgagagtgcaccataaaattgtaaacgttaatattttgttaaaattcgcgttaaatttttgttaaatcagctcattttttaaccaataggccgaaatcggcaaaatcccttataaatcaaaagaatagcccgagatagggttgagtgttgttccagtttggaacaagagtccactattaaagaacgtggactccaacgtcaaagggcgaaaaaccgtctatcagggcgatggcccactacgtgaaccatcacccaaatcaagttttttggggtcgaggtgccgtaaagcactaaatcggaaccctaaagggagcccccgatttagagcttgacggggaaagccggcgaacgtggcgagaaaggaagggaagaaagcgaaaggagcgggcgctagggcgctggcaagtgtagcggtcacgctgcgcgtaaccaccacacccgccgcgcttaatgcgccgctacagggcgcgtactatggttgctttgacgtatgcggtgtgaaataccgcacagatgcgtaaggagaaaataccgcatcaggcgccattcgccattcaggctgcgcaactgttgggaagggcgatcggtgcgggcctcttcgctattacgccagctggcgaaagggggatgtgctgcaaggcgattaagttgggtaacgccagggttttcccagtcacgacgttgtaaaacgacggccagtgccaagcttaccaaacagagaatccgtgagttacgataaaaggcgaaggagcaattgaagtcgcacgggtagaaggtgtgaatctcgagtgcgagcccgaagcacaaactcgagaaagccttctgccaacatgtcttccgtatttgatgagtacgaacagctcctcgcggctcagactcgccccaatggagctcatggagggggagaaaaagggagtaccttaaaagtagacgtcccggtattcactcttaacagtgatgacccagaagatagatggagctttgtggtattctgcctccggattgctgttagcgaagatgccaacaaaccactcaggcaaggtgctctcatatctcttttatgctcccactcacaggtaatgaggaaccatgttgcccttgcagggaaacagaatgaagccacattggccgtgcttgagattgatggctttgccaacggcacgccccagttcaacaataggagtggagtgtctgaagagagagcacagagatttgcgatgatagcaggatctctccctcgggcatgcagcaacggaaccccgttcgtcacagccggggccgaagatgatgcaccagaagacatcaccgataccctggagaggatcctctctatccaggctcaagtatgggtcacagtagcaaaagccatgactgcgtatgagactgcagatgagtcggaaacaaggcgaatcaataagtatatgcagcaaggcagggtccaaaagaaatacatcctctaccccgtatgcaggagcacaatccaactcacgatcagacagtctcttgcagtccgcatctttttggttagcgagctcaagagaggccgcaacacggcaggtggtacctctacttattataacctggtaggggacgtagactcatacatcaggaataccgggcttactgcattcttcttgacactcaagtacggaatcaacaccaagacatcagcccttgcacttagtagcctctcaggcgacatccagaagatgaagcagctcatgcgtttgtatcggatgaaaggagataatgcgccgtacatgacattacttggtgatagtgaccagatgagctttgcgcctgccgagtatgcacaactttactcctttgccatgggtatggcatcagtcctagataaaggtactgggaaataccaatttgccagggactttatgagcacatcattctggagacttggagtagagtacgctcaggctcagggaagtagcattaacgaggatatggctgccgagctaaagctaaccccagcagcaaggaggggcctggcagctgctgcccaacgggtctccgaggagaccagcagcatagacatgcctactcaacaagtcggagtcctcactgggcttagcgagggggggtcccaagctctacaaggcggatcgaatagatcgcaagggcaaccagaagccggggatggggagacccaattcctggatctgatgagagcggtagcaaatagcatgagggaggcgccaaactctgcacagggcactccccaatcggggcctcccccaactcctgggccatcccaagataacgacaccgactgggggtattgatggacaaaacccagcctgcttccacaaaaacatcccaatgccctcacccgtagtcgacccctcgatttgcggctctatatgaccacaccctcaaacaaacatccccctctttcctccctccccctgctgtacaactacgtacgccctagataccacaggcacaatgcggctcactaacaatcaaaacagagccgagggaattagaaaaaagtacgggtagaagagggatattcagagatcagggcaagtctcccgagtctctgctctctcctctacctgatagaccaggacaaacatggccacctttacagatgcagagatcgacgagctatttgagacaagtggaactgtcattgacaacataattacagcccagggtaaaccagcagagactgttggaaggagtgcaatcccacaaggcaagaccaaggtgctgagcgcagcatgggagaagcatgggagcatccagccaccggccagtcaagacaaccccgatcgacaggacagatctgacaaacaaccatccacacccgagcaaacgaccccgcatgacagcccgccggccacatccgccgaccagccccccacccaggccacagacgaagccgtcgacacacagctcaggaccggagcaagcaactctctgctgttgatgcttgacaagctcagcaataaatcgtccaatgctaaaaagggcccatggtcgagcccccaagaggggaatcaccaacgtccgactcaacagcaggggagtcaacccagtcgcggaaacagtcaggaaagaccgcagaaccaagtcaaggccgcccctggaaaccagggcacagacgtgaacacagcatatcatggacaatgggaggagtcacaactatcagctggtgcaacccctcatgctctccgatcaaggcagagccaagacaatacccttgtatctgcggatcatgtccagccacctgtagactttgtgcaagcgatgatgtctatgatggaggcgatatcacagagagtaagtaaggttgactatcagctagatcttgtcttgaaacagacatcctccatccctatgatgcggtccgaaatccaacagctgaaaacatctgttgcagtcatggaagccaacttgggaatgatgaagattctggatcccggttgtgccaacatttcatctctgagtgatctacgggcagttgcccgatctcacccggttttagtttcaggccctggagacccctctccctatgtgacacaaggaggcgaaatggcacttaataaactttcgcaaccagtgccacatccatctgaattgattaaacccgccactgcatgcgggcctgatataggagtggaaaaggacactgtccgtgcattgatcatgtcacgcccaatgcacccgagttcttcagccaagctcctaagcaagttagatgcagccgggtcgatcgaggaaatcaggaaaatcaagcgccttgctctaaatggctaattactactgccacacgtagcgggtccctgtccactcggcatcacacggaatctgcaccgagttcccccccgcggacccaaggtccaactctccaagcggcaatcctctctcgcttcctcagccccactgaatgatcgcgtaaccgtaattaatctagctacatttaagattaagaaaaaatacgggtagaattggagtgccccaattgtgccaagatggactcatctaggacaattgggctgtactttgattctgcccattcttctagcaacctgttagcatttccgatcgtcctacaagacacaggagatgggaagaagcaaatcgccccgcaatataggatccagcgccttgacttgtggactgatagtaaggaggactcagtattcatcaccacctatggattcatctttcaagttgggaatgaagaagccaccgtcggcatgatcgatgataaacccaagcgcgagttactttccgctgcgatgctctgcctaggaagcgtcccaaataccggagaccttattgagctggcaagggcctgtctcactatgatagtcacatgcaagaagagtgcaactaatactgagagaatggttttctcagtagtgcaggcaccccaagtgctgcaaagctgtagggttgtggcaaacaaatactcatcagtgaatgcagtcaagcacgtgaaagcgccagagaagattcccgggagtggaaccctagaatacaaggtgaactttgtctccttgactgtggtaccgaagagggatgtctacaagatcccagctgcagtattgaaggtttctggctcgagtctgtacaatcttgcgctcaatgtcactattaatgtggaggtagacccgaggagtcctttggttaaatctctgtctaagtctgacagcggatactatgctaacctcttcttgcatattggacttatgaccactgtagataggaaggggaagaaagtgacatttgacaagctggaaaagaaaataaggagccttgatctatctgtcgggctcagtgatgtgctcgggccttccgtgttggtaaaagcaagaggtgcacggactaagcttttggcacctttcttctctagcagtgggacagcctgctatcccatagcaaatgcttctcctcaggtggccaagatactctggagtcaaaccgcgtgcctgcggagcgttaaaatcattatccaagcaggtacccaacgcgctgtcgcagtgaccgccgaccacgaggttacctctactaagctggagaaggggcacacccttgccaaatacaatccttttaagaaataagctgcgtctctgagattgcgctccgcccactcacccagatcatcatgacacaaaaaactaatctgtcttgattatttacagttagtttacctgtctatcaagttagaaaaaacacgggtagaagattctggatcccggttggcgccctccaggtgcaagatgggctccagaccttctaccaagaacccagcacctatgatgctgactatccgggttgcgctggtactgagttgcatctgtccggcaaactccattgatggcaggcctcttgcagctgcaggaattgtggttacaggagacaaagccgtcaacatatacacctcatcccagacaggatcaatcatagttaagctcctcccgaatctgcccaaggataaggaggcatgtgcgaaagcccccttggatgcatacaacaggacattgaccactttgctcaccccccttggtgactctatccgtaggatacaagagtctgtgactacatctggagggcggagacagaggcgctttataggcgccattattggcggtgtggctcttggggttgcaactgccgcacaaataacagcggccgcagctctgatacaagccaaacaaaatgctgccaacatcctccgacttaaagagagcattgccgcaaccaatgaggctgtgcatgaggtcactgacggattatcgcaactagcagtggcagttgggaagatgcagcagtttgttaatgaccaatttaataaaacagctcaggaattagactgcatcaaaattgcacagcaagttggtgtagagctcaacctgtacctaaccgaattgactacagtattcggaccacaaatcacttcacctgctttaaacaagctgactattcaggcactttacaatctagctggtggaaatatggattacttattgactaagttaggtgtagggaacaatcaactcagctcattaatcggtagcggcttaatcaccggtaaccctattctatacgactcacagactcaactcttgggtatacaggtaactctaccttcagtcgggaacctaaataatatgcgtgccacctacttggaaaccttatccgtaagcacaaccaggggatttgcctcggcacttgtcccaaaagtggtgacacaggtcggttctgtgatagaagaacttgacacctcatactgtatagaaactgacttagatttatattgtacaagaatagtaacgttccctatgtcccctggtatttattcctgcttgagcggcaatacgtcggcctgtatgtactcaaagaccgaaggcgcacttactacaccatacatgactatcaaaggttcagtcatcgccaactgcaagatgacaacatgtagatgtgtaaaccccccgggtatcatatcgcaaaactatggagaagccgtgtctctaatagataaacaatcatgcaatgttttatccttaggcgggataactttaaggctcagtggggaattcgatgtaacttatcagaagaatatctcaatacaagattctcaagtaataataacaggcaatcttgatatctcaactgagcttgggaatgtcaacaactcgatcagtaatgctttgaataagttagaggaaagcaacagaaaactagacaaagtcaatgtcaaactgactagcacatctgctctcattacctatatcgttttgactatcatatctcttgtttttggtatacttagcctgattctagcatgctacctaatgtacaagcaaaaggcgcaacaaaagaccttattatggcttgggaataatactctagatcagatgagagccactacaaaaatgtgaacacagatgaggaacgaaggtttccctaatagtaatttgtgtgaaagttctggtagtctgtcagttcagagagttaagaaaaaactaccggttgtagatgaccaaaggacgatatacgggtagaacggtaagagaggccgcccctcaattgcgagccaggcttcacaacctccgttctaccgcttcaccgacaacagtcctcaatcatggaccgcgccgttagccaagttgcgttagagaatgatgaaagagaggcaaaaaatacatggcgcttgatattccggattgcaatcttattcttaacagtagtgaccttggctatatctgtagcctcccttttatatagcatgggggctagcacacctagcgatcttgtaggcataccgactaggatttccagggcagaagaaaagattacatctacacttggttccaatcaagatgtagtagataggatatataagcaagtggcccttgagtctccgttggcattgttaaatactgagaccacaattatgaacgcaataacatctctctcttatcagattaatggagctgcaaacaacagtgggtggggggcacctatccatgacccagattatataggggggataggcaaagaactcattgtagatgatgctagtgatgtcacatcattctatccctctgcatttcaagaacatctgaattttatcccggcgcctactacaggatcaggttgcactcgaataccctcatttgacatgagtgctacccattactgctacacccataatgtaatattgtctggatgcagagatcactcacattcatatcagtatttagcacttggtgtgctccggacatctgcaacagggagggtattcttttctactctgcgttccatcaacctggacgacacccaaaatcggaagtcttgcagtgtgagtgcaactcccctgggttgtgatatgctgtgctcgaaagtcacggagacagaggaagaagattataactcagctgtccctacgcggatggtacatgggaggttagggttcgacggccagtaccacgaaaaggacctagatgtcacaacattattcggggactgggtggccaactacccaggagtagggggtggatcttttattgacagccgcgtatggttctcagtctacggagggttaaaacccaattcacccagtgacactgtacaggaagggaaatatgtgatatacaagcgatacaatgacacatgcccagatgagcaagactaccagattcgaatggccaagtcttcgtataagcctggacggtttggtgggaaacgcatacagcaggctatcttatctatcaaggtgtcaacatccttaggcgaagacccggtactgactgtaccgcccaacacagtcacactcatgggggccgaaggcagaattctcacagtagggacatctcatttcttgtatcaacgagggtcatcatacttctctcccgcgttattatatcctatgacagtcagcaacaaaacagccactcttcatagtccttatacattcaatgccttcactcggccaggtagtatcccttgccaggcttcagcaagatgccccaactcgtgtgttactggagtctatacagatccatatcccctaatcttctatagaaaccacaccttgcgaggggtattcgggacaatgcttgatggtgtacaagcaagacttaaccctgcgtctgcagtattcgatagcacatcccgcagtcgcattactcgagtgagttcaagcagtaccaaagcagcatacacaacatcaacttgttttaaagtggtcaagactaataagacctattgtctcagcattgctgaaatatctaatactctcttcggagaattcagaatcgtcccgttactagttgagatcctcaaagatgacggggttagagaagccaggtctggctagttgagtcaattataaaggagttggaaagatggcattgtatcacctatcttctgcgacatcaagaatcaaaccgaatgccggcgcgtgctcgaattccatgttgccagttgaccacaatcagccagtgctcatgcgatcagattaagccttgtcaatagtctcttgattaagaaaaaatgtaagtggcaatgagatacaaggcaaaacagctcatggttaacaatacgggtaggacatggcgagctccggtcctgaaagggcagagcatcagattatcctaccagagtcacacctgtcttcaccattggtcaagcacaaactactctattactggaaattaactgggctaccgcttcctgatgaatgtgacttcgaccacctcattctcagccgacaatggaaaaaaatacttgaatcggcctctcctgatactgagagaatgataaaactcggaagggcagtacaccaaactcttaaccacaattccagaataaccggagtgctccaccccaggtgtttagaagaactggctaatattgaggtcccagattcaaccaacaaatttcggaagattgagaagaagatccaaattcacaacacgagatatggagaactgttcacaaggctgtgtacgcatatagagaagaaactgctggggtcatcttggtctaacaatgtcccccggtcagaggagttcagcagcattcgtacggatccggcattctggtttcactcaaaatggtccacagccaagtttgcatggctccatataaaacagatccagaggcatctgatggtggcagctaggacaaggtctgcggccaacaaattggtgatgctaacccataaggtaggccaagtctttgtcactcctgaacttgtcgttgtgacgcatacgaatgagaacaagttcacatgtcttacccaggaacttgtattgatgtatgcagatatgatggagggcagagatatggtcaacataatatcaaccacggcggtgcatctcagaagcttatcagagaaaattgatgacattttgcggttaatagacgctctggcaaaagacttgggtaatcaagtctacgatgttgtatcactaatggagggatttgcatacggagctgtccagctactcgagccgtcaggtacatttgcaggagatttcttcgcattcaacctgcaggagcttaaagacattctaattggcctcctccccaatgatatagcagaatccgtgactcatgcaatcgctactgtattctctggtttagaacagaatcaagcagctgagatgttgtgtctgttgcgtctgtggggtcacccactgcttgagtcccgtattgcagcaaaggcagtcaggagccaaatgtgcgcaccgaaaatggtagactttgatatgatccttcaggtactgtctttcttcaagggaacaatcatcaacgggtacagaaagaagaatgcaggtgtgtggccgcgagtcaaagtggatacaatatatgggaaggtcattgggcaactacatgcagattcagcagagatttcacacgatatcatgttgagagagtataagagtttatctgcacttgaatttgagccatgtatagaatatgaccctgtcaccaacctgagcatgttcctaaaagacaaggcaatcgcacaccccaacgataattggcttgcctcgtttaggcggaaccttctctccgaagaccagaagaaacatgtaaaagaagcaacttcgactaatcgcctcttgatagagtttttagagtcaaatgattttgatccatataaagagatggaatatctgacgacccttgagtaccttagagatgacaatgtggcagtatcatactcgctcaaggagaaggaagtgaaagttaatggacggatcttcgctaagctgacaaagaagttaaggaactgtcaggtgatggcggaagggatcctagccgatcagattgcacctttctttcagggaaatggagtcattcaggatagcatatccttgaccaagagtatgctagcgatgagtcaactgtcttttaacagcaataagaaacgtatcactgactgtaaagaaagagtatcttcaaaccgcaatcatgatccgaaaagcaagaaccgtcggagagttgcaaccttcataacaactgacctgcaaaagtactgtcttaattggagatatcagacaatcaaattgttcgctcatgccatcaatcagttgatgggcctacctcacttcttcgaatggattcacctaagactgatggacactacgatgttcgtaggagaccctttcaatcctccaagtgaccctactgactgtgacctctcaagagtccctaatgatgacatatatattgtcagtgccagagggggtatcgaaggattatgccagaagctatggacaatgatctcaattgctgcaatccaacttgctgcagctagatcgcattgtcgtgttgcctgtatggtacagggtgataatcaagtaatagcagtaacgagagaggtaagatcagacgactctccggagatggtgttgacacagttgcatcaagccagtgataatttcttcaaggaattaattcatgtcaatcatttgattggccataatttgaaggatcgtgaaaccatcaggtcagacacattcttcatatacagcaaacgaatcttcaaagatggagcaatcctcagtcaagtcctcaaaaattcatctaaattagtgctagtgtcaggtgatctcagtgaaaacaccgtaatgtcctgtgccaacattgcctctactgtagcacggctatgcgagaacgggcttcccaaagacttctgttactatttaaactatataatgagttgtgtgcagacatactttgactctgagttctccatcaccaacaattcgcaccccgatcttaatcagtcgtggattgaggacatctcttttgtgcactcatatgttctgactcctgcccaattagggggactgagtaaccttcaatactcaaggctctacactagaaatatcggtgacccggggactactgcttttgcagagatcaagcgactagaagcagtgggattactgagtcctaacattatgactaatatcttaactaggccgcctgggaatggagattgggccagtctgtgcaacgacccatactctttcaattttgagactgttgcaagcccaaatattgttcttaagaaacatacgcaaagagtcctatttgaaacttgttcaaatcccttattgtctggagtgcacacagaggataatgaggcagaagagaaggcattggctgaattcttgcttaatcaagaggtgattcatccccgcgttgcgcatgccatcatggaggcaagctctgtaggtaggagaaagcaaattcaagggcttgttgacacaacaaacaccgtaattaagattgcgcttactaggaggccattaggcatcaagaggctgatgcggatagtcaattattctagcatgcatgcaatgctgtttagagacgatgttttttcctccagtagatccaaccaccccttagtctcttctaatatgtgttctctgacactggcagactatgcacggaatagaagctggtcacctttgacgggaggcaggaaaatactgggtgtatctaatcctgatacgatagaactcgtagagggtgagattcttagtgtaagcggagggtgtacaagatgtgacagcggagatgaacaatttacttggttccatcttccaagcaatatagaattgaccgatgacaccagcaagaatcctccgatgagggtaccatatctcgggtcaaagacacaggagaggagagctgcctcacttgcaaaaatagctcatatgtcgccacatgtaaaggctgccctaagggcatcatccgtgttgatctgggcttatggggataatgaagtaaattggactgctgctcttacgattgcaaaatctcggtgtaatgtaaacttagagtatcttcggttactgtcccctttacccacggctgggaatcttcaacatagactagatgatggtataactcagatgacattcacccctgcatctctctacagggtgtcaccttacattcacatatccaatgattctcaaaggctgttcactgaagaaggagtcaaagaggggaatgtggtttaccaacagatcatgctcttgggtttatctctaatcgaatcgatctttccaatgacaacaaccaggacatatgatgagatcacactgcacctacatagtaaatttagttgctgtatcagagaagcacctgttgcggttcctttcgagctacttggggtggtaccggaactgaggacagtgacctcaaataagtttatgtatgatcctagccctgtatcggagggagactttgcgagacttgacttagctatcttcaagagttatgagcttaatctggagtcatatcccacgatagagctaatgaacattctttcaatatccagcgggaagttgattggccagtctgtggtttcttatgatgaagatacctccataaagaatgacgccataatagtgtatgacaatacccgaaattggatcagtgaagctcagaattcagatgtggtccgcctatttgaatatgcagcacttgaagtgctcctcgactgttcttaccaactctattacctgagagtaagaggcctggacaatattgtcttatatatgggtgatttatacaagaatatgccaggaattctactttccaacattgcagctacaatatctcatcccgtcattcattcaaggttacatgcagtgggcctggtcaaccatgacggatcacaccaacttgcagatacggattttatcgaaatgtctgcaaaactattagtatcttgcacccgacgtgtgatctccggcttatattcaggaaataagtatgatctgctgttcccatctgtcttagatgataacctgaatgagaagatgcttcagctgatatcccggttatgctgtctgtacacggtactctttgctacaacaagagaaatcccgaaaataagaggcttaactgcagaagagaaatgttcaatactcactgagtatttactgtcggatgctgtgaaaccattacttagccccgatcaagtgagctctatcatgtctcctaacataattacattcccagctaatctgtactacatgtctcggaagagcctcaatttgatcagggaaagggaggacagggatactatcctggcgttgttgttcccccaagagccattattagagttcccttctgtgcaagatattggtgctcgagtgaaagatccattcacccgacaacctgcggcatttttgcaagagttagatttgagtgctccagcaaggtatgacgcattcacacttagtcagattcatcctgaactcacatctccaaatccggaggaagactacttagtacgatacttgttcagagggatagggactgcatcttcctcttggtataaggcatctcatctcctttctgtacccgaggtaagatgtgcaagacacgggaactccttatacttagctgaagggagcggagccatcatgagtcttctcgaactgcatgtaccacatgaaactatctattacaatacgctcttttcaaatgagatgaaccccccgcaacgacatttcgggccgaccccaactcagtttttgaattcggttgtttataggaatctacaggcggaggtaacatgcaaagatggatttgtccaagagttccgtccattatggagagaaaatacagaggaaagcgacctgacctcagataaagtagtggggtatattacatctgcagtgccctacagatctgtatcattgctgcattgtgacattgaaattcctccagggtccaatcaaagcttactagatcaactagctatcaatttatctctgattgccatgcattctgtaagggagggcggggtagtaatcatcaaagtgttgtatgcaatgggatactactttcatctactcatgaacttgtttgctccgtgttccacaaaaggatatattctctctaatggttatgcatgtcgaggagatatggagtgttacctggtatttgtcatgggttacctgggcgggcctacatttgtacatgaggtggtgaggatggcgaaaactctggtgcagcggcacggtacgcttttgtctaaatcagatgagatcacactgaccaggttattcacctcacagcggcagcgtgtgacagacatcctatccagtcctttaccaagattaataaagtacttgaggaagaatattgacactgcgctgattgaagccgggggacagcccgtccgtccattctgtgcggagagtctggtgagcacgctagcgaacataactcagataacccagatcatcgctagtcacattgacacagttatccggtctgtgatatatatggaagctgagggtgatctcgctgacacagtatttctatttaccccttacaatctctctactgacgggaaaaagaggacatcacttaaacagtgcacgagacagatcctagaggttacaatactaggtcttagagtcgaaaatctcaataaaataggcgatataatcagcctagtgcttaaaggcatgatctccatggaggaccttatcccactaaggacatacttgaagcatagtacctgccctaaatatttgaaggctgtcctaggtattaccaaactcaaagaaatgtttacagacacttctgtactgtacttgactcgtgctcaacaaaaattctacatgaaaactataggcaatgcagtcaaaggatattacagtaactgtgactcttaacgaaaatcacatattaataggctccttttttggccaattgtattcttgttgatttaatcatattatgttagaaaaaagttgaaccctgactccttaggactcgaattcgaactcaaataaatgtcttaaaaaaaggttgcgcacaattattcttgagtgtagtctcgtcattcaccaaatctttgtttggtgcgcgcagatctgtcatgatgatcattgcaattggatccatatatagggcccgggttataattacctcaggtcgacgtcccatggccattcgaattcgtaatcatggtcatagctgtttcctgtgtgaaattgttatccgctcacaattccacacaacatacgagccggaagcataaagtgtaaagcctggggtgcctaatgagtgagctaactcacattaattgcgttgcgctcactgcccgctttccagtcgggaaacctgtcgtgccagctgcattaatgaatcggccaacgcgcggggagaggcggtttgcgtattgggcgc

SEQ ID NO: 7 - protein, 6 aa, SARS-CoV2
NFLPRP

SEQ ID NO: 8 - protein, 6 aa, SARS-CoV2
TFLARG

SEQ ID NO: 9 - protein, 6 aa, SARS-CoV2
RPSKRP

SEQ ID NO: 10 - protein, 6 aa, SARS-CoV2
LFLPRV

SEQ ID NO: 11 - protein, 1288 aa, SARS-CoV-2
MFVFLVLLPLVSSQCVNLTTRTQLPPAYTNSFTRGVYYPDKVFRSSVLHSTQDLFLPFFSNVTWFHAIHVSGTNGTKRFDNPVLPFNDGVYFASTEKSNIIRGWIFGTTLDSKTQSLLIVNNATNVVIKVCEFQFCNDPFLGVYYHKNNKSWMESEFRVYSSANNCTFEYVSQPFLMDLEGKQGNFKNLREFVFKNIDGYFKIYSKHTPINLVRDLPQGFSALEPLVDLPIGINITRFQTLLALHRSYLTPGDSSSGWTAGAAAYYVGYLQPRTFLLKYNENGTITDAVDCALDPLSETKCTLKSFTVEKGIYQTSNFRVQPTESIVRFPNITNLCPFGEVFNATRFASVYAWNRKRISNCVADYSVLYNSASFSTFKCYGVSPTKLNDLCFTNVYADSFVIRGDEVRQIAPGQTGKIADYNYKLPDDFTGCVIAWNSNNLDSKVGGNYNYLYRLFRKSNLKPFERDISTEIYQAGSTPCNGVEGFNCYFPLQSYGFQPTNGVGYQPYRVVVLSFELLHAPATVCGPKKSTNLVKNKCVNFNFNGLTGTGVLTESNKKFLPFQQFGRDIADTTDAVRDPQTLEILDITPCSFGGVSVITPGTNTSNQVAVLYQDVNCTEVPVAIHADQLTPTWRVYSTGSNVFQTRAGCLIGAEHVNNSYECDIPIGAGICASYQTQTNSPGSASSVASQSIIAYTMSLGAENSVAYSNNSIAIPTNFTISVTTEILPVSMTKTSVDCTMYICGDSTECSNLLLQYGSFCTQLNRALTGIAVEQDKNTQEVFAQVKQIYKTPPIKDFGGFNFSQILPDPSKPSKRSPIEDLLFNKVTLADAGFIKQYGDCLGDIAARDLICAQKFNGLTVLPPLLTDEMIAQYTSALLAGTITSGWTFGAGPALQIPFPMQMAYRFNGIGVTQNVLYENQKLIANQFNSAIGKIQDSLSSTPSALGKLQDVVNQNAQALNTLVKQLSSNFGAISSVLNDILSRLDPPEAEVQIDRLITGRLQSLQTYVTQQLIRAAEIRASANLAATKMSECVLGQSKRVDFCGKGYHLMSFPQSAPHGVVFLHVTYVPAQEKNFTTAPAICHDGKAHFPREGVFVSNGTHWFVTQRNFYEPQIITTDNTFVSGNCDVVIGIVNNTVYDPLQPELDSFKEELDKYFKNHTSPDVDLGDISGINASVVNIQKEIDRLNEVAKNLNESLIDLQELGKYEQGSGYIPEAPRDGQAYVRKDGEWVLLSTFLGRSLEVLFQGPGHHHHHHHHSAWSHPQFEKGGGSGGGGSGGSAWSHPQFEK

SEQ ID NO: 12 - protein, 1288 aa, SARS-CoV-2; identical to SEQ ID NO: 11

SEQ ID NO: 13 - protein, 1288 aa, SARS-CoV-2; identical to SEQ ID NO: 11

SEQ ID NO: 14 - DNA, 18394 bp, NDV LaSota
tcttccgcttcctcgctcactgactcgctgcgctcggtcgttcggctgcggcgagcggtatcagctcactcaaaggcggtaatacggttatccacagaatcaggggataacgcaggaaagaacatgtgagcaaaaggccagcaaaaggccaggaaccgtaaaaaggccgcgttgctggcgtttttccataggctccgcccccctgacgagcatcacaaaaatcgacgctcaagtcagaggtggcgaaacccgacaggactataaagataccaggcgtttccccctggaagctccctcgtgcgctctcctgttccgaccctgccgcttaccggatacctgtccgcctttctcccttcgggaagcgtggcgctttctcatagctcacgctgtaggtatctcagttcggtgtaggtcgttcgctccaagctgggctgtgtgcacgaaccccccgttcagcccgaccgctgcgccttatccggtaactatcgtcttgagtccaacccggtaagacacgacttatcgccactggcagcagccactggtaacaggattagcagagcgaggtatgtaggcggtgctacagagttcttgaagtggtggcctaactacggctacactagaagaacagtatttggtatctgcgctctgctgaagccagttaccttcggaaaaagagttggtagctcttgatccggcaaacaaaccaccgctggtagcggtggtttttttgtttgcaagcagcagattacgcgcagaaaaaaaggatctcaagaagatcctttgatcttttctacggggtctgacgctcagtggaacgaaaactcacgttaagggattttggtcatgagattatcaaaaaggatcttcacctagatccttttaaattaaaaatgaagttttaaatcaatctaaagtatatatgagtaaacttggtctgacagttaccaatgcttaatcagtgaggcacctatctcagcgatctgtctatttcgttcatccatagttgcctgactccccgtcgtgtagataactacgatacgggagggcttaccatctggccccagtgctgcaatgataccgcgagacccacgctcaccggctccagatttatcagcaataaaccagccagccggaagggccgagcgcagaagtggtcctgcaactttatccgcctccatccagtctattaattgttgccgggaagctagagtaagtagttcgccagttaatagtttgcgcaacgttgttgccattgctacaggcatcgtggtgtcacgctcgtcgtttggtatggcttcattcagctccggttcccaacgatcaaggcgagttacatgatcccccatgttgtgcaaaaaagcggttagctccttcggtcctccgatcgttgtcagaagtaagttggccgcagtgttatcactcatggttatggcagcactgcataattctcttactgtcatgccatccgtaagatgcttttctgtgactggtgagtactcaaccaagtcattctgagaatagtgtatgcggcgaccgagttgctcttgcccggcgtcaatacgggataataccgcgccacatagcagaactttaaaagtgctcatcattggaaaacgttcttcggggcgaaaactctcaaggatcttaccgctgttgagatccagttcgatgtaacccactcgtgcacccaactgatcttcagcatcttttactttcaccagcgtttctgggtgagcaaaaacaggaaggcaaaatgccgcaaaaaagggaataagggcgacacggaaatgttgaatactcatactcttcctttttcaatattattgaagcatttatcagggttattgtctcatgagcggatacatatttgaatgtatttagaaaaataaacaaataggggttccgcgcacatttccccgaaaagtgccacctgacgtctaagaaaccattattatcatgacattaacctataaaaataggcgtatcacgaggccctttcgtctcgcgcgtttcggtgatgacggtgaaaacctctgacacatgcagctcccggagacggtcacagcttgtctgtaagcggatgccgggagcagacaagcccgtcagggcgcgtcagcgggtgttggcgggtgtcggggctggcttaactatgcggcatcagagcagattgtactgagagtgcaccataaaattgtaaacgttaatattttgttaaaattcgcgttaaatttttgttaaatcagctcattttttaaccaataggccgaaatcggcaaaatcccttataaatcaaaagaatagcccgagatagggttgagtgttgttccagtttggaacaagagtccactattaaagaacgtggactccaacgtcaaagggcgaaaaaccgtctatcagggcgatggcccactacgtgaaccatcacccaaatcaagttttttggggtcgaggtgccgtaaagcactaaatcggaaccctaaagggagcccccgatttagagcttgacggggaaagccggcgaacgtggcgagaaaggaagggaagaaagcgaaaggagcgggcgctagggcgctggcaagtgtagcggtcacgctgcgcgtaaccaccacacccgccgcgcttaatgcgccgctacagggcgcgtactatggttgctttgacgtatgcggtgtgaaataccgcacagatgcgtaaggagaaaataccgcatcaggcgccattcgccattcaggctgcgcaactgttgggaagggcgatcggtgcgggcctcttcgctattacgccagctggcgaaagggggatgtgctgcaaggcgattaagttgggtaacgccagggttttcccagtcacgacgttgtaaaacgacggccagtgccaagcttaccaaacagagaatccgtgagttacgataaaaggcgaaggagcaattgaagtcgcacgggtagaaggtgtgaatctcgagtgcgagcccgaagcacaaactcgagaaagccttctgccaacatgtcttccgtatttgatgagtacgaacagctcctcgcggctcagactcgccccaatggagctcatggagggggagaaaaagggagtaccttaaaagtagacgtcccggtattcactcttaacagtgatgacccagaagatagatggagctttgtggtattctgcctccggattgctgttagcgaagatgccaacaaaccactcaggcaaggtgctctcatatctcttttatgctcccactcacaggtaatgaggaaccatgttgcccttgcagggaaacagaatgaagccacattggccgtgcttgagattgatggctttgccaacggcacgccccagttcaacaataggagtggagtgtctgaagagagagcacagagatttgcgatgatagcaggatctctccctcgggcatgcagcaacggaaccccgttcgtcacagccggggccgaagatgatgcaccagaagacatcaccgataccctggagaggatcctctctatccaggctcaagtatgggtcacagtagcaaaagccatgactgcgtatgagactgcagatgagtcggaaacaaggcgaatcaataagtatatgcagcaaggcagggtccaaaagaaatacatcctctaccccgtatgcaggagcacaatccaactcacgatcagacagtctcttgcagtccgcatctttttggttagcgagctcaagagaggccgcaacacggcaggtggtacctctacttattataacctggtaggggacgtagactcatacatcaggaataccgggcttactgcattcttcttgacactcaagtacggaatcaacaccaagacatcagcccttgcacttagtagcctctcaggcgacatccagaagatgaagcagctcatgcgtttgtatcggatgaaaggagataatgcgccgtacatgacattacttggtgatagtgaccagatgagctttgcgcctgccgagtatgcacaactttactcctttgccatgggtatggcatcagtcctagataaaggtactgggaaataccaatttgccagggactttatgagcacatcattctggagacttggagtagagtacgctcaggctcagggaagtagcattaacgaggatatggctgccgagctaaagctaaccccagcagcaaggaggggcctggcagctgctgcccaacgggtctccgaggagaccagcagcatagacatgcctactcaacaagtcggagtcctcactgggcttagcgagggggggtcccaagctctacaaggcggatcgaatagatcgcaagggcaaccagaagccggggatggggagacccaattcctggatctgatgagagcggtagcaaatagcatgagggaggcgccaaactctgcacagggcactccccaatcggggcctcccccaactcctgggccatcccaagataacgacaccgactgggggtattgatggacaaaacccagcctgcttccacaaaaacatcccaatgccctcacccgtagtcgacccctcgatttgcggctctatatgaccacaccctcaaacaaacatccccctctttcctccctccccctgctgtacaactacgtacgccctagataccacaggcacaatgcggctcactaacaatcaaaacagagccgagggaattagaaaaaagtacgggtagaagagggatattcagagatcagggcaagtctcccgagtctctgctctctcctctacctgatagaccaggacaaacatggccacctttacagatgcagagatcgacgagctatttgagacaagtggaactgtcattgacaacataattacagcccagggtaaaccagcagagactgttggaaggagtgcaatcccacaaggcaagaccaaggtgctgagcgcagcatgggagaagcatgggagcatccagccaccggccagtcaagacaaccccgatcgacaggacagatctgacaaacaaccatccacacccgagcaaacgaccccgcatgacagcccgccggccacatccgccgaccagccccccacccaggccacagacgaagccgtcgacacacagctcaggaccggagcaagcaactctctgctgttgatgcttgacaagctcagcaataaatcgtccaatgctaaaaagggcccatggtcgagcccccaagaggggaatcaccaacgtccgactcaacagcaggggagtcaacccagtcgcggaaacagtcaggaaagaccgcagaaccaagtcaaggccgcccctggaaaccagggcacagacgtgaacacagcatatcatggacaatgggaggagtcacaactatcagctggtgcaacccctcatgctctccgatcaaggcagagccaagacaatacccttgtatctgcggatcatgtccagccacctgtagactttgtgcaagcgatgatgtctatgatggaggcgatatcacagagagtaagtaaggttgactatcagctagatcttgtcttgaaacagacatcctccatccctatgatgcggtccgaaatccaacagctgaaaacatctgttgcagtcatggaagccaacttgggaatgatgaagattctggatcccggttgtgccaacatttcatctctgagtgatctacgggcagttgcccgatctcacccggttttagtttcaggccctggagacccctctccctatgtgacacaaggaggcgaaatggcacttaataaactttcgcaaccagtgccacatccatctgaattgattaaacccgccactgcatgcgggcctgatataggagtggaaaaggacactgtccgtgcattgatcatgtcacgcccaatgcacccgagttcttcagccaagctcctaagcaagttagatgcagccgggtcgatcgaggaaatcaggaaaatcaagcgccttgctctaaatggctaattactactgccacacgtagcgggtccctgtccactcggcatcacacggaatctgcaccgagttcccccccgcggacccaaggtccaactctccaagcggcaatcctctctcgcttcctcagccccactgaatgatcgcgtaaccgtaattaatctagctacatttaagattaagaaaaaatacgggtagaattggagtgccccaattgtgccaagatggactcatctaggacaattgggctgtactttgattctgcccattcttctagcaacctgttagcatttccgatcgtcctacaagacacaggagatgggaagaagcaaatcgccccgcaatataggatccagcgccttgacttgtggactgatagtaaggaggactcagtattcatcaccacctatggattcatctttcaagttgggaatgaagaagccaccgtcggcatgatcgatgataaacccaagcgcgagttactttccgctgcgatgctctgcctaggaagcgtcccaaataccggagaccttattgagctggcaagggcctgtctcactatgatagtcacatgcaagaagagtgcaactaatactgagagaatggttttctcagtagtgcaggcaccccaagtgctgcaaagctgtagggttgtggcaaacaaatactcatcagtgaatgcagtcaagcacgtgaaagcgccagagaagattcccgggagtggaaccctagaatacaaggtgaactttgtctccttgactgtggtaccgaagagggatgtctacaagatcccagctgcagtattgaaggtttctggctcgagtctgtacaatcttgcgctcaatgtcactattaatgtggaggtagacccgaggagtcctttggttaaatctctgtctaagtctgacagcggatactatgctaacctcttcttgcatattggacttatgaccactgtagataggaaggggaagaaagtgacatttgacaagctggaaaagaaaataaggagccttgatctatctgtcgggctcagtgatgtgctcgggccttccgtgttggtaaaagcaagaggtgcacggactaagcttttggcacctttcttctctagcagtgggacagcctgctatcccatagcaaatgcttctcctcaggtggccaagatactctggagtcaaaccgcgtgcctgcggagcgttaaaatcattatccaagcaggtacccaacgcgctgtcgcagtgaccgccgaccacgaggttacctctactaagctggagaaggggcacacccttgccaaatacaatccttttaagaaataagctgcgtctctgagattgcgctccgcccactcacccagatcatcatgacacaaaaaactaatctgtcttgattatttacagttagtttacctgtctatcaagttagaaaaaacacgggtagaagattctggatcccggttggcgccctccaggtgcaagatgggctccagaccttctaccaagaacccagcacctatgatgctgactatccgggttgcgctggtactgagttgcatctgtccggcaaactccattgatggcaggcctcttgcagctgcaggaattgtggttacaggagacaaagccgtcaacatatacacctcatcccagacaggatcaatcatagttaagctcctcccgaatctgcccaaggataaggaggcatgtgcgaaagcccccttggatgcatacaacaggacattgaccactttgctcaccccccttggtgactctatccgtaggatacaagagtctgtgactacatctggagggcggagacagaggcgctttataggcgccattattggcggtgtggctcttggggttgcaactgccgcacaaataacagcggccgcagctctgatacaagccaaacaaaatgctgccaacatcctccgacttaaagagagcattgccgcaaccaatgaggctgtgcatgaggtcactgacggattatcgcaactagcagtggcagttgggaagatgcagcagtttgttaatgaccaatttaataaaacagctcaggaattagactgcatcaaaattgcacagcaagttggtgtagagctcaacctgtacctaaccgaattgactacagtattcggaccacaaatcacttcacctgctttaaacaagctgactattcaggcactttacaatctagctggtggaaatatggattacttattgactaagttaggtgtagggaacaatcaactcagctcattaatcggtagcggcttaatcaccggtaaccctattctatacgactcacagactcaactcttgggtatacaggtaactgccccttcagtcgggaacctaaataatatgcgtgccacctacttggaaaccttatccgtaagcacaaccaggggatttgcctcggcacttgtcccaaaagtggtgacacaggtcggttctgtgatagaagaacttgacacctcatactgtatagaaactgacttagatttatattgtacaagaatagtaacgttccctatgtcccctggtatttattcctgcttgagcggcaatacgtcggcctgtatgtactcaaagaccgaaggcgcacttactacaccatacatgactatcaaaggttcagtcatcgccaactgcaagatgacaacatgtagatgtgtaaaccccccgggtatcatatcgcaaaactatggagaagccgtgtctctaatagataaacaatcatgcaatgttttatccttaggcgggataactttaaggctcagtggggaattcgatgtaacttatcagaagaatatctcaatacaagattctcaagtaataataacaggcaatcttgatatctcaactgagcttgggaatgtcaacaactcgatcagtaatgctttgaataagttagaggaaagcaacagaaaactagacaaagtcaatgtcaaactgactagcacatctgctctcattacctatatcgttttgactatcatatctcttgtttttggtatacttagcctgattctagcatgctacctaatgtacaagcaaaaggcgcaacaaaagaccttattatggcttgggaataatactctagatcagatgagagccactacaaaaatgtgaacacagatgaggaacgaaggtttccctaatagtaatttgtgtgaaagttctggtagtctgtcagttcagagagttaagaaaaaactaccggttgtagatgaccaaaggacgatatacgggtagaacggtaagagaggccgcccctcaattgcgagccaggcttcacaacctccgttctaccgcttcaccgacaacagtcctcaatcatggaccgcgccgttagccaagttgcgttagagaatgatgaaagagaggcaaaaaatacatggcgcttgatattccggattgcaatcttattcttaacagtagtgaccttggctatatctgtagcctcccttttatatagcatgggggctagcacacctagcgatcttgtaggcataccgactaggatttccagggcagaagaaaagattacatctacacttggttccaatcaagatgtagtagataggatatataagcaagtggcccttgagtctccgttggcattgttaaatactgagaccacaattatgaacgcaataacatctctctcttatcagattaatggagctgcaaacaacagtgggtggggggcacctatccatgacccagattatataggggggataggcaaagaactcattgtagatgatgctagtgatgtcacatcattctatccctctgcatttcaagaacatctgaattttatcccggcgcctactacaggatcaggttgcactcgaataccctcatttgacatgagtgctacccattactgctacacccataatgtaatattgtctggatgcagagatcactcacattcatatcagtatttagcacttggtgtgctccggacatctgcaacagggagggtattcttttctactctgcgttccatcaacctggacgacacccaaaatcggaagtcttgcagtgtgagtgcaactcccctgggttgtgatatgctgtgctcgaaagtcacggagacagaggaagaagattataactcagctgtccctacgcggatggtacatgggaggttagggttcgacggccagtaccacgaaaaggacctagatgtcacaacattattcggggactgggtggccaactacccaggagtagggggtggatcttttattgacagccgcgtatggttctcagtctacggagggttaaaacccaattcacccagtgacactgtacaggaagggaaatatgtgatatacaagcgatacaatgacacatgcccagatgagcaagactaccagattcgaatggccaagtcttcgtataagcctggacggtttggtgggaaacgcatacagcaggctatcttatctatcaaggtgtcaacatccttaggcgaagacccggtactgactgtaccgcccaacacagtcacactcatgggggccgaaggcagaattctcacagtagggacatctcatttcttgtatcaacgagggtcatcatacttctctcccgcgttattatatcctatgacagtcagcaacaaaacagccactcttcatagtccttatacattcaatgccttcactcggccaggtagtatcccttgccaggcttcagcaagatgccccaactcgtgtgttactggagtctatacagatccatatcccctaatcttctatagaaaccacaccttgcgaggggtattcgggacaatgcttgatggtgtacaagcaagacttaaccctgcgtctgcagtattcgatagcacatcccgcagtcgcattactcgagtgagttcaagcagtaccaaagcagcatacacaacatcaacttgttttaaagtggtcaagactaataagacctattgtctcagcattgctgaaatatctaatactctcttcggagaattcagaatcgtcccgttactagttgagatcctcaaagatgacggggttagagaagccaggtctggctagttgagtcaattataaaggagttggaaagatggcattgtatcacctatcttctgcgacatcaagaatcaaaccgaatgccggcgcgtgctcgaattccatgttgccagttgaccacaatcagccagtgctcatgcgatcagattaagccttgtcaatagtctcttgattaagaaaaaatgtaagtggcaatgagatacaaggcaaaacagctcatggttaacaatacgggtaggacatggcgagctccggtcctgaaagggcagagcatcagattatcctaccagagtcacacctgtcttcaccattggtcaagcacaaactactctattactggaaattaactgggctaccgcttcctgatgaatgtgacttcgaccacctcattctcagccgacaatggaaaaaaatacttgaatcggcctctcctgatactgagagaatgataaaactcggaagggcagtacaccaaactcttaaccacaattccagaataaccggagtgctccaccccaggtgtttagaagaactggctaatattgaggtcccagattcaaccaacaaatttcggaagattgagaagaagatccaaattcacaacacgagatatggagaactgttcacaaggctgtgtacgcatatagagaagaaactgctggggtcatcttggtctaacaatgtcccccggtcagaggagttcagcagcattcgtacggatccggcattctggtttcactcaaaatggtccacagccaagtttgcatggctccatataaaacagatccagaggcatctgatggtggcagctaggacaaggtctgcggccaacaaattggtgatgctaacccataaggtaggccaagtctttgtcactcctgaacttgtcgttgtgacgcatacgaatgagaacaagttcacatgtcttacccaggaacttgtattgatgtatgcagatatgatggagggcagagatatggtcaacataatatcaaccacggcggtgcatctcagaagcttatcagagaaaattgatgacattttgcggttaatagacgctctggcaaaagacttgggtaatcaagtctacgatgttgtatcactaatggagggatttgcatacggagctgtccagctactcgagccgtcaggtacatttgcaggagatttcttcgcattcaacctgcaggagcttaaagacattctaattggcctcctccccaatgatatagcagaatccgtgactcatgcaatcgctactgtattctctggtttagaacagaatcaagcagctgagatgttgtgtctgttgcgtctgtggggtcacccactgcttgagtcccgtattgcagcaaaggcagtcaggagccaaatgtgcgcaccgaaaatggtagactttgatatgatccttcaggtactgtctttcttcaagggaacaatcatcaacgggtacagaaagaagaatgcaggtgtgtggccgcgagtcaaagtggatacaatatatgggaaggtcattgggcaactacatgcagattcagcagagatttcacacgatatcatgttgagagagtataagagtttatctgcacttgaatttgagccatgtatagaatatgaccctgtcaccaacctgagcatgttcctaaaagacaaggcaatcgcacaccccaacgataattggcttgcctcgtttaggcggaaccttctctccgaagaccagaagaaacatgtaaaagaagcaacttcgactaatcgcctcttgatagagtttttagagtcaaatgattttgatccatataaagagatggaatatctgacgacccttgagtaccttagagatgacaatgtggcagtatcatactcgctcaaggagaaggaagtgaaagttaatggacggatcttcgctaagctgacaaagaagttaaggaactgtcaggtgatggcggaagggatcctagccgatcagattgcacctttctttcagggaaatggagtcattcaggatagcatatccttgaccaagagtatgctagcgatgagtcaactgtcttttaacagcaataagaaacgtatcactgactgtaaagaaagagtatcttcaaaccgcaatcatgatccgaaaagcaagaaccgtcggagagttgcaaccttcataacaactgacctgcaaaagtactgtcttaattggagatatcagacaatcaaattgttcgctcatgccatcaatcagttgatgggcctacctcacttcttcgaatggattcacctaagactgatggacactacgatgttcgtaggagaccctttcaatcctccaagtgaccctactgactgtgacctctcaagagtccctaatgatgacatatatattgtcagtgccagagggggtatcgaaggattatgccagaagctatggacaatgatctcaattgctgcaatccaacttgctgcagctagatcgcattgtcgtgttgcctgtatggtacagggtgataatcaagtaatagcagtaacgagagaggtaagatcagacgactctccggagatggtgttgacacagttgcatcaagccagtgataatttcttcaaggaattaattcatgtcaatcatttgattggccataatttgaaggatcgtgaaaccatcaggtcagacacattcttcatatacagcaaacgaatcttcaaagatggagcaatcctcagtcaagtcctcaaaaattcatctaaattagtgctagtgtcaggtgatctcagtgaaaacaccgtaatgtcctgtgccaacattgcctctactgtagcacggctatgcgagaacgggcttcccaaagacttctgttactatttaaactatataatgagttgtgtgcagacatactttgactctgagttctccatcaccaacaattcgcaccccgatcttaatcagtcgtggattgaggacatctcttttgtgcactcatatgttctgactcctgcccaattagggggactgagtaaccttcaatactcaaggctctacactagaaatatcggtgacccggggactactgcttttgcagagatcaagcgactagaagcagtgggattactgagtcctaacattatgactaatatcttaactaggccgcctgggaatggagattgggccagtctgtgcaacgacccatactctttcaattttgagactgttgcaagcccaaatattgttcttaagaaacatacgcaaagagtcctatttgaaacttgttcaaatcccttattgtctggagtgcacacagaggataatgaggcagaagagaaggcattggctgaattcttgcttaatcaagaggtgattcatccccgcgttgcgcatgccatcatggaggcaagctctgtaggtaggagaaagcaaattcaagggcttgttgacacaacaaacaccgtaattaagattgcgcttactaggaggccattaggcatcaagaggctgatgcggatagtcaattattctagcatgcatgcaatgctgtttagagacgatgttttttcctccagtagatccaaccaccccttagtctcttctaatatgtgttctctgacactggcagactatgcacggaatagaagctggtcacctttgacgggaggcaggaaaatactgggtgtatctaatcctgatacgatagaactcgtagagggtgagattcttagtgtaagcggagggtgtacaagatgtgacagcggagatgaacaatttacttggttccatcttccaagcaatatagaattgaccgatgacaccagcaagaatcctccgatgagggtaccatatctcgggtcaaagacacaggagaggagagctgcctcacttgcaaaaatagctcatatgtcgccacatgtaaaggctgccctaagggcatcatccgtgttgatctgggcttatggggataatgaagtaaattggactgctgctcttacgattgcaaaatctcggtgtaatgtaaacttagagtatcttcggttactgtcccctttacccacggctgggaatcttcaacatagactagatgatggtataactcagatgacattcacccctgcatctctctacagggtgtcaccttacattcacatatccaatgattctcaaaggctgttcactgaagaaggagtcaaagaggggaatgtggtttaccaacagatcatgctcttgggtttatctctaatcgaatcgatctttccaatgacaacaaccaggacatatgatgagatcacactgcacctacatagtaaatttagttgctgtatcagagaagcacctgttgcggttcctttcgagctacttggggtggtaccggaactgaggacagtgacctcaaataagtttatgtatgatcctagccctgtatcggagggagactttgcgagacttgacttagctatcttcaagagttatgagcttaatctggagtcatatcccacgatagagctaatgaacattctttcaatatccagcgggaagttgattggccagtctgtggtttcttatgatgaagatacctccataaagaatgacgccataatagtgtatgacaatacccgaaattggatcagtgaagctcagaattcagatgtggtccgcctatttgaatatgcagcacttgaagtgctcctcgactgttcttaccaactctattacctgagagtaagaggcctggacaatattgtcttatatatgggtgatttatacaagaatatgccaggaattctactttccaacattgcagctacaatatctcatcccgtcattcattcaaggttacatgcagtgggcctggtcaaccatgacggatcacaccaacttgcagatacggattttatcgaaatgtctgcaaaactattagtatcttgcacccgacgtgtgatctccggcttatattcaggaaataagtatgatctgctgttcccatctgtcttagatgataacctgaatgagaagatgcttcagctgatatcccggttatgctgtctgtacacggtactctttgctacaacaagagaaatcccgaaaataagaggcttaactgcagaagagaaatgttcaatactcactgagtatttactgtcggatgctgtgaaaccattacttagccccgatcaagtgagctctatcatgtctcctaacataattacattcccagctaatctgtactacatgtctcggaagagcctcaatttgatcagggaaagggaggacagggatactatcctggcgttgttgttcccccaagagccattattagagttcccttctgtgcaagatattggtgctcgagtgaaagatccattcacccgacaacctgcggcatttttgcaagagttagatttgagtgctccagcaaggtatgacgcattcacacttagtcagattcatcctgaactcacatctccaaatccggaggaagactacttagtacgatacttgttcagagggatagggactgcatcttcctcttggtataaggcatctcatctcctttctgtacccgaggtaagatgtgcaagacacgggaactccttatacttagctgaagggagcggagccatcatgagtcttctcgaactgcatgtaccacatgaaactatctattacaatacgctcttttcaaatgagatgaaccccccgcaacgacatttcgggccgaccccaactcagtttttgaattcggttgtttataggaatctacaggcggaggtaacatgcaaagatggatttgtccaagagttccgtccattatggagagaaaatacagaggaaagcgacctgacctcagataaagtagtggggtatattacatctgcagtgccctacagatctgtatcattgctgcattgtgacattgaaattcctccagggtccaatcaaagcttactagatcaactagctatcaatttatctctgattgccatgcattctgtaagggagggcggggtagtaatcatcaaagtgttgtatgcaatgggatactactttcatctactcatgaacttgtttgctccgtgttccacaaaaggatatattctctctaatggttatgcatgtcgaggagatatggagtgttacctggtatttgtcatgggttacctgggcgggcctacatttgtacatgaggtggtgaggatggcgaaaactctggtgcagcggcacggtacgcttttgtctaaatcagatgagatcacactgaccaggttattcacctcacagcggcagcgtgtgacagacatcctatccagtcctttaccaagattaataaagtacttgaggaagaatattgacactgcgctgattgaagccgggggacagcccgtccgtccattctgtgcggagagtctggtgagcacgctagcgaacataactcagataacccagatcatcgctagtcacattgacacagttatccggtctgtgatatatatggaagctgagggtgatctcgctgacacagtatttctatttaccccttacaatctctctactgacgggaaaaagaggacatcacttaaacagtgcacgagacagatcctagaggttacaatactaggtcttagagtcgaaaatctcaataaaataggcgatataatcagcctagtgcttaaaggcatgatctccatggaggaccttatcccactaaggacatacttgaagcatagtacctgccctaaatatttgaaggctgtcctaggtattaccaaactcaaagaaatgtttacagacacttctgtactgtacttgactcgtgctcaacaaaaattctacatgaaaactataggcaatgcagtcaaaggatattacagtaactgtgactcttaacgaaaatcacatattaataggctccttttttggccaattgtattcttgttgatttaatcatattatgttagaaaaaagttgaaccctgactccttaggactcgaattcgaactcaaataaatgtcttaaaaaaaggttgcgcacaattattcttgagtgtagtctcgtcattcaccaaatctttgtttggtgcgcgcagatctgtcatgatgatcattgcaattggatccatatatagggcccgggttataattacctcaggtcgacgtcccatggccattcgaattcgtaatcatggtcatagctgtttcctgtgtgaaattgttatccgctcacaattccacacaacatacgagccggaagcataaagtgtaaagcctggggtgcctaatgagtgagctaactcacattaattgcgttgcgctcactgcccgctttccagtcgggaaacctgtcgtgccagctgcattaatgaatcggccaacgcgcggggagaggcggtttgcgtattgggcgc